European Patent Specification EP 3 298 025 B1, published February 11, 2026. Title: New amino acid sequences with microbicidal activity derived from Naja atra cardiotoxin 1 (CTX-1). Applicant: Università degli Studi di Parma. The sequence listing filed with the application follows.

SEQUENCE LISTING (10 sequences)

SEQ ID NO: 1 - protein, 20 aa, Unknown
  None
KLIPILSKTIPAIKNLFYKI

SEQ ID NO: 2 - protein, 20 aa, Unknown
  None
KLIWILSKTIPAIKNLFYKI

SEQ ID NO: 3 - protein, 20 aa, Unknown
  None
KLIPIASKTIPAGKNLFYKI

SEQ ID NO: 4 - protein, 20 aa, Unknown
  None
KLIPIASKTIPAGKNLIYKI

SEQ ID NO: 5 - protein, 20 aa, Unknown
  None
KLIPIASKTIPAGKNLLYKI

SEQ ID NO: 6 - protein, 20 aa, Unknown
  None
KLIPIASKTIPAGKNLVYKI

SEQ ID NO: 7 - protein, 20 aa, Unknown
  None
KLIFILSKTIPAIKNLFYKI

SEQ ID NO: 8 - protein, 20 aa, Unknown
  None
KLILILSKTIPAIKNLFYKI

SEQ ID NO: 9 - protein, 20 aa, Unknown
  None
KLIYILSKTIPAIKNLFYKI

SEQ ID NO: 10 - protein, 20 aa, Unknown
  None
KLIPIASKTCPAGKNLCYKI